European Patent Application EP 4 782 837 A1, published July 29, 2026. Title: COMPOSITION FOR PREDICTING CETUXIMAB RESPONSIVENESS IN CANCER. Applicant: KOREA INSTITUTE OF SCIENCE AND TECHNOLOGY. Application KR. The sequence listing filed with the application follows.

SEQUENCE LISTING (2 sequences)

SEQ ID NO: 1 - protein, 8 aa, synthetic construct
  source 1..8: note = C-probe
GFLGGKGG

SEQ ID NO: 2 - protein, 8 aa, synthetic construct
  source 1..8: note = C2 probe
GGFGGKGG